European Patent Application EP 4 711 463 A1, published March 18, 2026. Title: Lipid Complex. Applicant: EISAI R & D Management Co., Ltd. Application JP. The sequence listing filed with the application follows.

SEQUENCE LISTING (31 sequences)

SEQ ID NO: 1 - protein, 429 aa, Human T-cell leukemia virus type 1
  source 1..429: note = Gag
MGQIFSRSASPIPRPPRGLAAHHWLNFLQAAYRLEPGPSSYDFHQLKKFLKIALETPVWICPINYSLLASLLPKGYPGRVNEILHILIQTQAQIPSRPAPPPPSSPTHDPPDSDPQIPPPYVEPTAPQVLPVMHPHGAPPNHRPWQMKDLQAIKQEVSQAAPGSPQFMQTIRLAVQQFDPTAKDLQDLLQYLCSSLVASLHHQQLDSLISEAETRGITGYNPLAGPLRVQANNPQQQGLRREYQQLWLAAFAALPGSAKDPSWASILQGLEEPYHAFVERLNIALDNGLPEGTPKDPILRSLAYSNANKECQKLLQARGHTNSPLGDMLRACQTWTPKDKTKVLVVQPKKPPPNQPCFRCGKAGHWSRDCTQPRPPPGPCPLCQDPTHWKRDCPRLKPTIPEPEPEEDALLLDLPADIPHPKNSIGGEV

SEQ ID NO: 2 - RNA, 1557 nt, Human T-cell leukemia virus type 1
  source 1..1557: mol_type = mRNA
aggaaataagagagaaaagaagagtaagaagaaatataagagccaccatgggccagatcttctctcgctctgcttctcctattcctcgccctcctcgcggacttgctgctcaccactggcttaacttcctgcaggctgcttaccgcctggaacctggccctagcagctacgacttccaccagctgaagaagttcctgaagatcgccctggagacccccgtgtggatctgccccatcaactacagcctgctggctagcctgctgcctaaaggctaccctggccgcgtgaacgagatcctgcacatcctgatccagacccaggcccagatcccttctcgccctgctcctcctcctccttcttctcctacccacgatccccccgatagcgatccccagatcccccctccttacgtggaacctaccgctcctcaggtgctgcctgtgatgcaccctcacggcgctcctcctaatcaccgcccttggcagatgaaggacctgcaggccatcaaacaggaagtgagccaggctgctcccggcagcccccagtttatgcagaccatccgcctggctgtgcagcagttcgatcccaccgctaaagatctgcaggacctgctgcagtacctgtgcagcagcctggtggctagcctgcaccaccagcagctggatagcctgatcagcgaagccgaaacccgcggcatcaccggctacaatcctctggctggccctctgcgcgtgcaggctaacaaccctcagcagcagggactgcgccgcgaataccagcagctgtggctggctgcttttgctgctctgcccggcagcgctaaagatcccagctgggctagcatcctgcagggcctggaagaaccctaccacgccttcgtggagcgcctgaacatcgccctggacaacggcctgcctgaaggcacccctaaagatcctatcctgcgcagcctggcctacagcaacgccaacaaggagtgccagaagctgctgcaggctcgcggacacaccaatagccctctgggagatatgctgcgcgcttgccagacctggacccccaaggacaagaccaaggtgctggtggtgcagcccaagaagcctcctcctaaccagccttgctttcgctgcggcaaagctggacactggagccgcgattgcacacagcctcgccctcctcctggaccttgccctctttgccaggatcctacccactggaagcgcgactgccctcgcctgaaacctaccatccctgaacctgaacctgaagaagacgctctgctgctggatctgcccgctgatatcccccaccccaagaacagcatcggcggcgaggtgtgataagctgccttctgcggggcttgccttctggccatgcccttcttctctcccttgcacctgtacctcttggtctttgaataaagcctgagtaggaaggcggaaaaaaaaaaaaaaaaaaaaaaaaaaaaaaaaaaaaaaaaaaaaaaaaaaaaaaaaaaaaaaaaaaaaaaaaaaaaaaaaaaaaaaaaaaaaaaaaaaaaaaaaaaaaaaaaaaaaaaaa

SEQ ID NO: 3 - RNA, 1287 nt, Human T-cell leukemia virus type 1
  source 1..1287: mol_type = mRNA
atgggccagatcttctctcgctctgcttctcctattcctcgccctcctcgcggacttgctgctcaccactggcttaacttcctgcaggctgcttaccgcctggaacctggccctagcagctacgacttccaccagctgaagaagttcctgaagatcgccctggagacccccgtgtggatctgccccatcaactacagcctgctggctagcctgctgcctaaaggctaccctggccgcgtgaacgagatcctgcacatcctgatccagacccaggcccagatcccttctcgccctgctcctcctcctccttcttctcctacccacgatccccccgatagcgatccccagatcccccctccttacgtggaacctaccgctcctcaggtgctgcctgtgatgcaccctcacggcgctcctcctaatcaccgcccttggcagatgaaggacctgcaggccatcaaacaggaagtgagccaggctgctcccggcagcccccagtttatgcagaccatccgcctggctgtgcagcagttcgatcccaccgctaaagatctgcaggacctgctgcagtacctgtgcagcagcctggtggctagcctgcaccaccagcagctggatagcctgatcagcgaagccgaaacccgcggcatcaccggctacaatcctctggctggccctctgcgcgtgcaggctaacaaccctcagcagcagggactgcgccgcgaataccagcagctgtggctggctgcttttgctgctctgcccggcagcgctaaagatcccagctgggctagcatcctgcagggcctggaagaaccctaccacgccttcgtggagcgcctgaacatcgccctggacaacggcctgcctgaaggcacccctaaagatcctatcctgcgcagcctggcctacagcaacgccaacaaggagtgccagaagctgctgcaggctcgcggacacaccaatagccctctgggagatatgctgcgcgcttgccagacctggacccccaaggacaagaccaaggtgctggtggtgcagcccaagaagcctcctcctaaccagccttgctttcgctgcggcaaagctggacactggagccgcgattgcacacagcctcgccctcctcctggaccttgccctctttgccaggatcctacccactggaagcgcgactgccctcgcctgaaacctaccatccctgaacctgaacctgaagaagacgctctgctgctggatctgcccgctgatatcccccaccccaagaacagcatcggcggcgaggtg

SEQ ID NO: 4 - protein, 353 aa, Human T-cell leukemia virus type 1
  source 1..353: note = Tax
MAHFPGFGQSLLFGYPVYVFGDCVQGDWCPISGGLCSARLHRHALLATCPEHQITWDPIDGRVIGSALQFLIPRLPSFPTQRTSKTLKVLTPPITHTTPNIPPSFLQAMRKYSPFRNGYMEPTLGQHLPTLSFPDPGLRPQNLYTLWGGSVVCMYLYQLSPPITWPLLPHVIFCHPGQLGAFLTNVPYKRIEELLYKISLTTGALIILPEDCLPTTLFQPARAPVTLTAWQNGLLPFHSTLTTPGLIWTFTDGTPMISGPCPKDGQPSLVLQSSSFIFHKFQTKAYHPSFLLSHGLIQYSSFHSLHLLFEEYTNIPISLLFNEKEADDNDHEPQISPGGLEPPSEKHFRETEV

SEQ ID NO: 5 - RNA, 1329 nt, Human T-cell leukemia virus type 1
  source 1..1329: mol_type = mRNA
aggaaataagagagaaaagaagagtaagaagaaatataagagccaccatggcccacttccccggctttggccagagcctgctgtttggctaccccgtgtacgtgttcggcgattgcgtgcagggcgattggtgccccatctctggaggactgtgctctgctcgccttcaccgccacgcacttcttgctacatgccctgagcaccagatcacctgggatcccatcgatggccgcgtgatcggcagcgctctgcagttcctgatccctcgcctgcctagctttcctacccagcgcaccagcaaaaccctgaaggtgctgacccctcctatcacccacaccacccctaacatccctcctagcttcctgcaggccatgcgcaagtacagccccttccgcaacggctacatggaacccaccctgggccagcacctgcctaccctgagctttcctgatcctggactgcgccctcagaatctgtacaccctgtggggaggaagcgtggtgtgcatgtacctgtaccagctgagccctcctatcacctggcctctgctgcctcacgtgatcttttgccaccctggccagctgggcgcttttctgaccaacgtgccttacaagcgcatcgaggagctgctgtacaagatcagcctgaccaccggcgccctgatcatcctgcccgaagattgcctgcccaccaccctgtttcagcctgctcgcgctcctgtgacactgacagcttggcagaacggcctgctgccttttcacagcaccctgaccacccctggcctgatctggaccttcaccgatggcacccccatgatcagcggcccttgccctaaagatggccagcctagcctggtgctgcagagcagcagcttcatcttccacaagttccagaccaaggcctaccaccccagcttcctgctgagccacggcctgatccagtacagcagcttccacagcctgcacctgctgttcgaggagtacaccaacatccccatcagcctgctgttcaacgagaaggaggccgacgacaacgaccacgagcctcagatcagccctggcggcctggaacctcctagcgaaaagcacttccgcgagaccgaggtgtgataagctgccttctgcggggcttgccttctggccatgcccttcttctctcccttgcacctgtacctcttggtctttgaataaagcctgagtaggaaggcggaaaaaaaaaaaaaaaaaaaaaaaaaaaaaaaaaaaaaaaaaaaaaaaaaaaaaaaaaaaaaaaaaaaaaaaaaaaaaaaaaaaaaaaaaaaaaaaaaaaaaaaaaaaaaaaaaaaaaaaa

SEQ ID NO: 6 - RNA, 1059 nt, Human T-cell leukemia virus type 1
  source 1..1059: mol_type = mRNA
atggcccacttccccggctttggccagagcctgctgtttggctaccccgtgtacgtgttcggcgattgcgtgcagggcgattggtgccccatctctggaggactgtgctctgctcgccttcaccgccacgcacttcttgctacatgccctgagcaccagatcacctgggatcccatcgatggccgcgtgatcggcagcgctctgcagttcctgatccctcgcctgcctagctttcctacccagcgcaccagcaaaaccctgaaggtgctgacccctcctatcacccacaccacccctaacatccctcctagcttcctgcaggccatgcgcaagtacagccccttccgcaacggctacatggaacccaccctgggccagcacctgcctaccctgagctttcctgatcctggactgcgccctcagaatctgtacaccctgtggggaggaagcgtggtgtgcatgtacctgtaccagctgagccctcctatcacctggcctctgctgcctcacgtgatcttttgccaccctggccagctgggcgcttttctgaccaacgtgccttacaagcgcatcgaggagctgctgtacaagatcagcctgaccaccggcgccctgatcatcctgcccgaagattgcctgcccaccaccctgtttcagcctgctcgcgctcctgtgacactgacagcttggcagaacggcctgctgccttttcacagcaccctgaccacccctggcctgatctggaccttcaccgatggcacccccatgatcagcggcccttgccctaaagatggccagcctagcctggtgctgcagagcagcagcttcatcttccacaagttccagaccaaggcctaccaccccagcttcctgctgagccacggcctgatccagtacagcagcttccacagcctgcacctgctgttcgaggagtacaccaacatccccatcagcctgctgttcaacgagaaggaggccgacgacaacgaccacgagcctcagatcagccctggcggcctggaacctcctagcgaaaagcacttccgcgagaccgaggtg

SEQ ID NO: 7 - protein, 206 aa, Human T-cell leukemia virus type 1
  source 1..206: note = HBZ
MAASGLFRCLPVSCPEDLLVEELVDGLLSLEEELKDKEEEEAVLDGLLSLEEESRGRLRRGPPGEKAPPRGETHRDRQRRAEEKRKRKKEREKEEEKQTAEYLKRKEEEKARRRRRAEKKAADVARRKQEEQERRERKWRQGAEKAKQHSARKEKMQELGIDGYTRQLEGEVESLEAERRKLLQEKEDLMGEVNYWQGRLEAMWLQ

SEQ ID NO: 8 - protein, 206 aa, Human T-cell leukemia virus type 1
  source 1..206: note = HBZ
MAASGLFRCLPVSCPEDLLVEELVDGLLSLEEELKDKEEEEAVLDGLLSLEEESRGRLRRGPPGEKAPPRGETHRDRQRRAEEKRKRKKEREKEEEKQIAEYLKRKEEEKARRRRRAEKKAADVARRKQEEQERRERKWRQGAEKAKQHSARKEKMQELGIDGYTRQLEGEVESLEAERRKLLQEKEDLMGEVNYWQGRLEAMWLQ

SEQ ID NO: 9 - RNA, 888 nt, Human T-cell leukemia virus type 1
  source 1..888: mol_type = mRNA
aggaaataagagagaaaagaagagtaagaagaaatataagagccaccatggctgctagcggcctgtttcgctgcctgcctgtgagctgccctgaagacctgctggtggaggaactggtggacggcctgctgagcctggaagaagaactgaaggacaaggaggaggaagaagccgtgctggacggcctgctgagcctggaagaagaatctcgcggacgccttcgccgcggacctcctggagaaaaagctcctcctagaggagaaacacacagagatagacaaagaaaagctgaggagaagcgcaagcgcaagaaggagcgcgagaaggaggaggagaagcagatcgccgagtacctgaagcgcaaagaagaagaaaaagctcgccgccgccgccgcgctgaaaaaaaagctgctgatgtggcccgccgcaaacaggaagaacaggaacgccgcgaacgcaaatggcgccagggcgctgaaaaagctaagcagcacagcgcccgcaaggagaagatgcaggaactgggcatcgacggctacacccgccagctggaaggcgaagtggaaagcctggaagccgaacgccgcaagctgctgcaggagaaggaggacctgatgggcgaggtgaactactggcagggccgcctggaagccatgtggctgcagtgataagctgccttctgcggggcttgccttctggccatgcccttcttctctcccttgcacctgtacctcttggtctttgaataaagcctgagtaggaaggcggaaaaaaaaaaaaaaaaaaaaaaaaaaaaaaaaaaaaaaaaaaaaaaaaaaaaaaaaaaaaaaaaaaaaaaaaaaaaaaaaaaaaaaaaaaaaaaaaaaaaaaaaaaaaaaaaaaaaaaaa

SEQ ID NO: 10 - RNA, 618 nt, Human T-cell leukemia virus type 1
  source 1..618: mol_type = mRNA
atggctgctagcggcctgtttcgctgcctgcctgtgagctgccctgaagacctgctggtggaggaactggtggacggcctgctgagcctggaagaagaactgaaggacaaggaggaggaagaagccgtgctggacggcctgctgagcctggaagaagaatctcgcggacgccttcgccgcggacctcctggagaaaaagctcctcctagaggagaaacacacagagatagacaaagaaaagctgaggagaagcgcaagcgcaagaaggagcgcgagaaggaggaggagaagcagatcgccgagtacctgaagcgcaaagaagaagaaaaagctcgccgccgccgccgcgctgaaaaaaaagctgctgatgtggcccgccgcaaacaggaagaacaggaacgccgcgaacgcaaatggcgccagggcgctgaaaaagctaagcagcacagcgcccgcaaggagaagatgcaggaactgggcatcgacggctacacccgccagctggaaggcgaagtggaaagcctggaagccgaacgccgcaagctgctgcaggagaaggaggacctgatgggcgaggtgaactactggcagggccgcctggaagccatgtggctgcag

SEQ ID NO: 11 - protein, 105 aa, Human T-cell leukemia virus type 1
  source 1..105: note = Gag p15
VVQPKKPPPNQPCFRCGKAGHWSRDCTQPRPPPGPCPLCQDPTHWKRDCPRLKPTIPEPEPEEDALLLDLPADIPHPKNLHRGGGLTSPPTLQQVLPNQDPASIL

SEQ ID NO: 12 - protein, 85 aa, Human T-cell leukemia virus type 1
  source 1..85: note = Gag p15
VVQPKKPPPNQPCFRCGKAGHWSRDCTQPRPPPGPCPLCQDPTHWKRDCPRLKPTIPEPEPEEDALLLDLPADIPHPKNSIGGEV

SEQ ID NO: 13 - protein, 130 aa, Human T-cell leukemia virus type 1
  source 1..130: note = Gag p19
MGQIFSRSASPIPRPPRGLAAHHWLNFLQAAYRLEPGPSSYDFHQLKKFLKIALETPVWICPINYSLLASLLPKGYPGRVNEILHILIQTQAQIPSRPAPPPPSSPTHDPPDSDPQIPPPYVEPTAPQVL

SEQ ID NO: 14 - protein, 214 aa, Human T-cell leukemia virus type 1
  source 1..214: note = Gag p24
PVMHPHGAPPNHRPWQMKDLQAIKQEVSQAAPGSPQFMQTIRLAVQQFDPTAKDLQDLLQYLCSSLVASLHHQQLDSLISEAETRGITGYNPLAGPLRVQANNPQQQGLRREYQQLWLAAFAALPGSAKDPSWASILQGLEEPYHAFVERLNIALDNGLPEGTPKDPILRSLAYSNANKECQKLLQARGHTNSPLGDMLRACQTWTPKDKTKVL

SEQ ID NO: 15 - RNA, 254 nt, Human T-cell leukemia virus type 1
  source 1..254: mol_type = mRNA
tggtgcagcccaagaagcctcctcctaaccagccttgctttcgctgcggcaaagctggacactggagccgcgattgcacacagcctcgccctcctcctggaccttgccctctttgccaggatcctacccactggaagcgcgactgccctcgcctgaaacctaccatccctgaacctgaacctgaagaagacgctctgctgctggatctgcccgctgatatcccccaccccaagaacagcatcggcggcgaggtg

SEQ ID NO: 16 - RNA, 387 nt, Human T-cell leukemia virus type 1
  source 1..387: mol_type = mRNA
ggccagatcttctctcgctctgcttctcctattcctcgccctcctcgcggacttgctgctcaccactggcttaacttcctgcaggctgcttaccgcctggaacctggccctagcagctacgacttccaccagctgaagaagttcctgaagatcgccctggagacccccgtgtggatctgccccatcaactacagcctgctggctagcctgctgcctaaaggctaccctggccgcgtgaacgagatcctgcacatcctgatccagacccaggcccagatcccttctcgccctgctcctcctcctccttcttctcctacccacgatccccccgatagcgatccccagatcccccctccttacgtggaacctaccgctcctcaggtgctg

SEQ ID NO: 17 - RNA, 643 nt, Human T-cell leukemia virus type 1
  source 1..643: mol_type = mRNA
cctgtgatgcaccctcacggcgctcctcctaatcaccgcccttggcagatgaaggacctgcaggccatcaaacaggaagtgagccaggctgctcccggcagcccccagtttatgcagaccatccgcctggctgtgcagcagttcgatcccaccgctaaagatctgcaggacctgctgcagtacctgtgcagcagcctggtggctagcctgcaccaccagcagctggatagcctgatcagcgaagccgaaacccgcggcatcaccggctacaatcctctggctggccctctgcgcgtgcaggctaacaaccctcagcagcagggactgcgccgcgaataccagcagctgtggctggctgcttttgctgctctgcccggcagcgctaaagatcccagctgggctagcatcctgcagggcctggaagaaccctaccacgccttcgtggagcgcctgaacatcgccctggacaacggcctgcctgaaggcacccctaaagatcctatcctgcgcagcctggcctacagcaacgccaacaaggagtgccagaagctgctgcaggctcgcggacacaccaatagccctctgggagatatgctgcgcgcttgccagacctggacccccaaggacaagaccaaggtgctgg

SEQ ID NO: 18 - DNA, 17 bp, synthetic construct
  source 1..17: mol_type = other DNA; note = T7 promoter
taatacgactcactata

SEQ ID NO: 19 - DNA, 41 bp, synthetic construct
  source 1..41: mol_type = other DNA; note = 5'UTR
aggaaataagagagaaaagaagagtaagaagaaatataaga

SEQ ID NO: 20 - skipped

SEQ ID NO: 21 - DNA, 100 bp, synthetic construct
  source 1..100: mol_type = other DNA; note = 3'UTR
taagctgccttctgcggggcttgccttctggccatgcccttcttctctcccttgcacctgtacctcttggtctttgaataaagcctgagtaggaaggcgg

SEQ ID NO: 22 - DNA, 1454 bp, Human T-cell leukemia virus type 1
  source 1..1454: mol_type = genomic DNA
taatacgactcactataaggaaataagagagaaaagaagagtaagaagaaatataagagccaccatgggccagatcttctctcgctctgcttctcctattcctcgccctcctcgcggacttgctgctcaccactggcttaacttcctgcaggctgcttaccgcctggaacctggccctagcagctacgacttccaccagctgaagaagttcctgaagatcgccctggagacccccgtgtggatctgccccatcaactacagcctgctggctagcctgctgcctaaaggctaccctggccgcgtgaacgagatcctgcacatcctgatccagacccaggcccagatcccttctcgccctgctcctcctcctccttcttctcctacccacgatccccccgatagcgatccccagatcccccctccttacgtggaacctaccgctcctcaggtgctgcctgtgatgcaccctcacggcgctcctcctaatcaccgcccttggcagatgaaggacctgcaggccatcaaacaggaagtgagccaggctgctcccggcagcccccagtttatgcagaccatccgcctggctgtgcagcagttcgatcccaccgctaaagatctgcaggacctgctgcagtacctgtgcagcagcctggtggctagcctgcaccaccagcagctggatagcctgatcagcgaagccgaaacccgcggcatcaccggctacaatcctctggctggccctctgcgcgtgcaggctaacaaccctcagcagcagggactgcgccgcgaataccagcagctgtggctggctgcttttgctgctctgcccggcagcgctaaagatcccagctgggctagcatcctgcagggcctggaagaaccctaccacgccttcgtggagcgcctgaacatcgccctggacaacggcctgcctgaaggcacccctaaagatcctatcctgcgcagcctggcctacagcaacgccaacaaggagtgccagaagctgctgcaggctcgcggacacaccaatagccctctgggagatatgctgcgcgcttgccagacctggacccccaaggacaagaccaaggtgctggtggtgcagcccaagaagcctcctcctaaccagccttgctttcgctgcggcaaagctggacactggagccgcgattgcacacagcctcgccctcctcctggaccttgccctctttgccaggatcctacccactggaagcgcgactgccctcgcctgaaacctaccatccctgaacctgaacctgaagaagacgctctgctgctggatctgcccgctgatatcccccaccccaagaacagcatcggcggcgaggtgtgataagctgccttctgcggggcttgccttctggccatgcccttcttctctcccttgcacctgtacctcttggtctttgaataaagcctgagtaggaaggcgg

SEQ ID NO: 23 - DNA, 1226 bp, Human T-cell leukemia virus type 1
  source 1..1226: mol_type = genomic DNA
taatacgactcactataaggaaataagagagaaaagaagagtaagaagaaatataagagccaccatggcccacttccccggctttggccagagcctgctgtttggctaccccgtgtacgtgttcggcgattgcgtgcagggcgattggtgccccatctctggaggactgtgctctgctcgccttcaccgccacgcacttcttgctacatgccctgagcaccagatcacctgggatcccatcgatggccgcgtgatcggcagcgctctgcagttcctgatccctcgcctgcctagctttcctacccagcgcaccagcaaaaccctgaaggtgctgacccctcctatcacccacaccacccctaacatccctcctagcttcctgcaggccatgcgcaagtacagccccttccgcaacggctacatggaacccaccctgggccagcacctgcctaccctgagctttcctgatcctggactgcgccctcagaatctgtacaccctgtggggaggaagcgtggtgtgcatgtacctgtaccagctgagccctcctatcacctggcctctgctgcctcacgtgatcttttgccaccctggccagctgggcgcttttctgaccaacgtgccttacaagcgcatcgaggagctgctgtacaagatcagcctgaccaccggcgccctgatcatcctgcccgaagattgcctgcccaccaccctgtttcagcctgctcgcgctcctgtgacactgacagcttggcagaacggcctgctgccttttcacagcaccctgaccacccctggcctgatctggaccttcaccgatggcacccccatgatcagcggcccttgccctaaagatggccagcctagcctggtgctgcagagcagcagcttcatcttccacaagttccagaccaaggcctaccaccccagcttcctgctgagccacggcctgatccagtacagcagcttccacagcctgcacctgctgttcgaggagtacaccaacatccccatcagcctgctgttcaacgagaaggaggccgacgacaacgaccacgagcctcagatcagccctggcggcctggaacctcctagcgaaaagcacttccgcgagaccgaggtgtgataagctgccttctgcggggcttgccttctggccatgcccttcttctctcccttgcacctgtacctcttggtctttgaataaagcctgagtaggaaggcgg

SEQ ID NO: 24 - DNA, 785 bp, Human T-cell leukemia virus type 1
  source 1..785: mol_type = genomic DNA
taatacgactcactataaggaaataagagagaaaagaagagtaagaagaaatataagagccaccatggctgctagcggcctgtttcgctgcctgcctgtgagctgccctgaagacctgctggtggaggaactggtggacggcctgctgagcctggaagaagaactgaaggacaaggaggaggaagaagccgtgctggacggcctgctgagcctggaagaagaatctcgcggacgccttcgccgcggacctcctggagaaaaagctcctcctagaggagaaacacacagagatagacaaagaaaagctgaggagaagcgcaagcgcaagaaggagcgcgagaaggaggaggagaagcagatcgccgagtacctgaagcgcaaagaagaagaaaaagctcgccgccgccgccgcgctgaaaaaaaagctgctgatgtggcccgccgcaaacaggaagaacaggaacgccgcgaacgcaaatggcgccagggcgctgaaaaagctaagcagcacagcgcccgcaaggagaagatgcaggaactgggcatcgacggctacacccgccagctggaaggcgaagtggaaagcctggaagccgaacgccgcaagctgctgcaggagaaggaggacctgatgggcgaggtgaactactggcagggccgcctggaagccatgtggctgcagtgataagctgccttctgcggggcttgccttctggccatgcccttcttctctcccttgcacctgtacctcttggtctttgaataaagcctgagtaggaaggcgg

SEQ ID NO: 25 - protein, 487 aa, Human T-cell leukemia virus type 1
  source 1..487: note = Env
GKFLATLILFFQFCPLIFGDYSPSCCTLTIGVSSYHSKPCNPAQPVCSWTLDLLALSADQALQPPCPNLVSYSSYHATYSLYLFPHWIKKPNRNGGGYYSASYSDPCSLKCPYLGCQSWTCPYTGAVSSPYWKFQHDVNFTQEVSRLNINLHFSKCGFPFSLLVDAPGYDPIWFLNTEPSQLPPTAPPLLPHSNLDHILEPSIPWKSKLLTLVQLTLQSTNYTCIVCIDRASLSTWHVLYSPNVSVPSSSSTPLLYPSLALPAPHLTLPFNWTHCFDPQIQAIVSSPCHNSLILPPFSLSPVPTLGSRSRRAVPVAVWLVSALAMGAGVAGGITGSMSLASGKSLLHEVDKDISQLTQAIVKNHKNLLKIAQYAAQNRRGLDLLFWEQGGLCKALQEQCCFLNITNSHVSILQERPPLENRVLTGWGLNWDLGLSQWAREALQTGITLVALLLLVILAGPCILRQLRHLPSRVRYPHYSLINPESSL

SEQ ID NO: 26 - DNA, 15 bp, synthetic construct
  source 1..15: mol_type = other DNA; note = cDNA synthesis primer for Gag
tgcaggatatgggcc

SEQ ID NO: 27 - DNA, 20 bp, synthetic construct
  source 1..20: mol_type = other DNA; note = primer set for Gag
agtacctttgctcctccctc

SEQ ID NO: 28 - DNA, 20 bp, synthetic construct
  source 1..20: mol_type = other DNA; note = primer set for Gag
taatacctcgggtttcggcc

SEQ ID NO: 29 - DNA, 27 bp, synthetic construct
  source 1..27: mol_type = other DNA; note = probe for Gag
ttccctccatcaccagctagatagcct

SEQ ID NO: 30 - DNA, 17 bp, synthetic construct
  source 1..17: mol_type = other DNA; note = primer set for Tax
ccgccgatcccaaagaa

SEQ ID NO: 31 - DNA, 19 bp, synthetic construct
  source 1..19: mol_type = other DNA; note = primer set for Tax
cctgtccaaaccctgggaa